European Patent Specification EP 3 423 090 B1, published August 30, 2023. Title: Novel Influenza Antigens. Applicant: GlaxoSmithKline Biologicals S.A. The sequence listing filed with the application follows.

SEQUENCE LISTING (11 sequences)

SEQ ID NO: 1 - protein, 588 aa, Artificial
  recombinant H5 haemagglutinin (ECD-TMD-foldon) Indo05
DQICIGYHANNSTEQVDTIMEKNVTVTHAQDILEKTHNGKLCDLDGVKPLILRDCSVAGWLLGNPMCDEFINVPEWSYIVEKANPTNDLCYPGSFNDYEELKHLLSRINHFEKIQIIPKSSWSDHEASSGBSSACPYLGSPSFFRNVVWLIKKNSTYPTIKKSYNNTNQEDLLVLWGIHHPNDAAEQTRLYQNPTTYISIGTSTLNQRLVPKIATRSKVNGQSGRMEFFWTILKPNDAINFESNGNFIAPEYAYKIVKKGDSAIMKSELEYGNCNTKCQTPMGAINSSPMFHNIHPLTIGECPKYBKSNRLVLATGLRNSPQRESRRKKRGLFGAIAGFIEGGWQGMVDGWYGYHHSNEQGSGYAADKESTQKAIDGVTNKVNSIIDKMNTQFEAVGREFNNLERRIENLNKKMEDGFLDVWTYNAELLVLMENERTLDFHDSNVKNLYDKVRLQLRDNAKELGNGCFEFYHKCDNECMESIRNGTYNYPQYSEEARLKREEISGVKLESIGTYQILSIYSTVASSLALAIMMAGLSLWMCSSGRLVPRGSPGSGYIPEAPRDGQAYVRKDGEWVLLSTFLGHHHHHH

SEQ ID NO: 2 - DNA, 1776 bp, Artificial
  recombinant H5 haemagglutinin (ECD-TMD-foldon)
gatcccggggatcagatttgcattggttaccatgcaaacaattcaacagagcaggttgacacaatcatggaaaagaacgttactgttacacatgcccaagacatactggaaaagacacacaacgggaagctctgcgatctagatggagtgaagcctctaattttaagagattgtagtgtagctggatggctcctcgggaacccaatgtgtgacgaattcatcaatgtaccggaatggtcttacatagtggagaaggccaatccaaccaatgacctctgttacccagggagtttcaacgactatgaagaactgaaacacctattgagcagaataaaccattttgagaaaattcaaatcatccccaaaagttcttggtccgatcatgaagcctcatcaggagtgagctcagcatgtccatacctgggaagtccctccttttttagaaatgtggtatggcttatcaaaaagaacagtacatacccaacaataaagaaaagctacaataataccaaccaagaagatcttttggtactgtggggaattcaccatcctaatgatgcggcagagcagacaaggctatatcaaaacccaaccacctatatttccattgggacatcaacactaaaccagagattggtaccaaaaatagctactagatccaaagtaaacgggcaaagtggaaggatggagttcttctggacaattttaaaacctaatgatgcaatcaacttcgagagtaatggaaatttcattgctccagaatatgcatacaaaattgtcaagaaaggggactcagcaattatgaaaagtgaattggaatatggtaactgcaacaccaagtgtcaaactccaatgggggcgataaactctagtatgccattccacaacatacaccctctcaccatcggggaatgccccaaatatgtgaaatcaaacagattagtccttgcaacagggctcagaaatagccctcaaagagagagcagaagaaaaaagagaggactatttggagctatagcaggttttatagagggaggatggcagggaatggtagatggttggtatgggtaccaccatagcaatgagcaggggagtgggtacgctgcagacaaagaatccactcaaaaggcaatagatggagtcaccaataaggtcaactcaatcattgacaaaatgaacactcagtttgaggccgttggaagggaatttaataacttagaaaggagaatagagaatttaaacaagaagatggaagacgggtttctagatgtctggacttataatgccgaacttctggttctcatggaaaatgagagaactctagactttcatgactcaaatgttaagaacctctacgacaaggtccgactacagcttagggataatgcaaaggagctgggtaacggttgtttcgagttctatcacaaatgtgataatgaatgtatggaaagtataagaaacggaacgtacaactatccgcagtattcagaagaagcaagactaaaaagagaggaaataagtggggtaaaattggaatcaataggaacttaccaaatactgtcaatttattcaacagtggcgagttccctagcactggcaatcatgatggctggtctatctttatggatgtgctccagcggccgcttggtccctcgtggaagcccaggctccggctacatccccgaggccccgcgcgacggccaggcctacgtgcgcaaggacggcgagtgggtgctgctgtccaccttcctgggacatcatcatcatcatcattga

SEQ ID NO: 3 - protein, 10 aa, Influenza Virus
NGSLQCRICI

SEQ ID NO: 4 - DNA, 30 bp, Influenza virus
aatggatcgttacaatgcagaatttgcatt

SEQ ID NO: 5 - protein, 38 aa, Influenza Virus
GVKLESIGTYQILSIYSTVASSLALAIMMAGLSLWMCS

SEQ ID NO: 6 - DNA, 114 bp, Influenza Virus
ggggtaaaattggaatcaataggaacttaccaaatactgtcaatttattcaacagtggcgagttccctagcactggcaatcatgatggctggtctatctttatggatgtgctcc

SEQ ID NO: 7 - protein, 504 aa, Influenza Virus
DQICIGYHANNSTEQVDTIMEKNVTVTHAQDILEKTHNGKLCDLDGVKPLILRDCSVAGWLLGNPMCDEFINVPEWSYIVEKANPTNDLCYPGSFNDYEELKHLLSRINHFEKIQIIPKSSWSDHEASSGBSSACPYLGSPSFFRNVVWLIKKNSTYPTIKKSYNNTNQEDLLVLWGIHHPNDAAEQTRLYQNPTTYISIGTSTLNQRLVPKIATRSKVNGQSGRMEFFWTILKPNDAINFESNGNFIAPEYAYKIVKKGDSAIMKSELEYGNCNTKCQTPMGAINSSMPFHNIHPLTIGECPKYVKSNRLVLATGLRNSPQRESRRKKRGLFGAIAGFIEGGWQGMVDGWYGYHHSNEQGSGYAADKESTQKAIDGVTNKVNSIIDKMNTQFEAVGREFNNLERRIENLNKKMEDGFLDVWTYNAELLVLMENERTLDFHDSNVKNLYDKVRLQLRDNAKELGNGCFEFYHKCDNECMESIRNGTYNYPQYSEEARLKREEIS

SEQ ID NO: 8 - DNA, 1521 bp, Influenza Virus
gatcccggggatcagatttgcattggttaccatgcaaacaattcaacagagcaggttgacacaatcatggaaaagaacgttactgttacacatgcccaagacatactggaaaagacacacaacgggaagctctgcgatctagatggagtgaagcctctaattttaagagattgtagtgtagctggatggctcctcgggaacccaatgtgtgacgaattcatcaatgtaccggaatggtcttacatagtggagaaggccaatccaaccaatgacctctgttacccagggagtttcaacgactatgaagaactgaaacacctattgagcagaataaaccattttgagaaaattcaaatcatccccaaaagttcttggtccgatcatgaagcctcatcaggagtgagctcagcatgtccatacctgggaagtccctccttttttagaaatgtggtatggcttatcaaaaagaacagtacatacccaacaataaagaaaagctacaataataccaaccaagaagatcttttggtactgtggggaattcaccatcctaatgatgcggcagagcagacaaggctatatcaaaacccaaccacctatatttccattgggacatcaacactaaaccagagattggtaccaaaaatagctactagatccaaagtaaacgggcaaagtggaaggatggagttcttctggacaattttaaaacctaatgatgcaatcaacttcgagagtaatggaaatttcattgctccagaatatgcatacaaaattgtcaagaaaggggactcagcaattatgaaaagtgaattggaatatggtaactgcaacaccaagtgtcaaactccaatgggggcgataaactctagtatgccattccacaacatacaccctctcaccatcggggaatgccccaaatatgtgaaatcaaacagattagtccttgcaacagggctcagaaatagccctcaaagagagagcagaagaaaaaagagaggactatttggagctatagcaggttttatagagggaggatggcagggaatggtagatggttggtatgggtaccaccatagcaatgagcaggggagtgggtacgctgcagacaaagaatccactcaaaaggcaatagatggagtcaccaataaggtcaactcaatcattgacaaaatgaacactcagtttgaggccgttggaagggaatttaataacttagaaaggagaatagagaatttaaacaagaagatggaagacgggtttctagatgtctggacttataatgccgaacttctggttctcatggaaaatgagagaactctagactttcatgactcaaatgttaagaacctctacgacaaggtccgactacagcttagggataatgcaaaggagctgggtaacggttgtttcgagttctatcacaaatgtgataatgaatgtatggaaagtataagaaacggaacgtacaactatccgcagtattcagaagaagcaagactaaaaagagaggaaataagt

SEQ ID NO: 9 - protein, 29 aa, Bacteriophage
GSGYIPEAPRDGQAYVRKDGEWVLLSTFL

SEQ ID NO: 10 - DNA, 87 bp, Bacteriophage
ggctccggctacatccccgaggccccgcgcgacggccaggcctacgtgcgcaaggacggcgagtgggtgctgctgtccaccttcctg

SEQ ID NO: 11 - protein, 564 aa, Influenza Virus
DQICIGYHANNSTEQVDTIMEKNVTVTHAQDILEKTHNGKLCDLDGVKPLILRDCSVAGWLLGNPMCDEFINVPEWSYIVEKANPTNDLCYPGSFNDYEELKHLLSRINHFEKIQIIPKSSWSDHEASSGBSSACPYLGSPSFFRNVVWLIKKNSTYPTIKKSYNNTNQEDLLVLWGIHHPNDAAEQTRLYQNPTTYISIGTSTLNQRLVPKIATRSKVNGQSGRMEFFWTILKPNDAINFESNGNFIAPEYAYKIVKKGDSAIMKSELEYGNCNTKCQTPMGAINSSMPFHNIHPLTIGECPKYVKSNRLVLATGLRNSPQRESRRKKRGLFGAIAGFIEGGWQGMVDGWYGYHHSNEQGSGYAADKESTQKAIDGVTNKVNSIIDKMNTQFEAVGREFNNLERRIENLNKKMEDGFLDVWTYNAELLVLMENERTLDFHDSNVKNLYDKVRLQLRDNAKELGNGCFEFYHKCDNECMESIRNGTYNYPQYSEEARLKREEISGVKLESIGTYQILSIYSTVASSLALAIMMAGLSTWMCSNGSLQCRICILVPRGSHHHHHH